European Patent Application EP 4 155 406 A1, published March 29, 2023. Title: MRNA OR MRNA COMPOSITION, AND PREPARATION METHOD THEREFOR AND APPLICATION THEREOF. Applicant: CANSINO (SHANGHAI) BIOTECHNOLOGIES CO., LTD. The sequence listing filed with the application follows.

SEQUENCE LISTING (19 sequences)

SEQ ID NO: 1 - protein, 1273 aa, Artificial Sequence
  wild-type full-length S protein
MFVFLVLLPLVSSQCVNLTTRTQLPPAYTNSFTRGVYYPDKVFRSSVLHSTQDLFLPFFSNVTWFHAIHVSGTNGTKRFDNPVLPFNDGVYFASTEKSNIIRGWIFGTTLDSKTQSLLIVNNATNVVIKVCEFQFCNDPFLGVYYHKNNKSWMESEFRVYSSANNCTFEYVSQPFLMDLEGKQGNFKNLREFVFKNIDGYFKIYSKHTPINLVRDLPQGFSALEPLVDLPIGINITRFQTLLALHRSYLTPGDSSSGWTAGAAAYYVGYLQPRTFLLKYNENGTITDAVDCALDPLSETKCTLKSFTVEKGIYQTSNFRVQPTESIVRFPNITNLCPFGEVFNATRFASVYAWNRKRISNCVADYSVLYNSASFSTFKCYGVSPTKLNDLCFTNVYADSFVIRGDEVRQIAPGQTGKIADYNYKLPDDFTGCVIAWNSNNLDSKVGGNYNYLYRLFRKSNLKPFERDISTEIYQAGSTPCNGVEGFNCYFPLQSYGFQPTNGVGYQPYRVVVLSFELLHAPATVCGPKKSTNLVKNKCVNFNFNGLTGTGVLTESNKKFLPFQQFGRDIADTTDAVRDPQTLEILDITPCSFGGVSVITPGTNTSNQVAVLYQDVNCTEVPVAIHADQLTPTWRVYSTGSNVFQTRAGCLIGAEHVNNSYECDIPIGAGICASYQTQTNSPRRARSVASQSIIAYTMSLGAENSVAYSNNSIAIPTNFTISVTTEILPVSMTKTSVDCTMYICGDSTECSNLLLQYGSFCTQLNRALTGIAVEQDKNTQEVFAQVKQIYKTPPIKDFGGFNFSQILPDPSKPSKRSFIEDLLFNKVTLADAGFIKQYGDCLGDIAARDLICAQKFNGLTVLPPLLTDEMIAQYTSALLAGTITSGWTFGAGAALQIPFAMQMAYRFNGIGVTQNVLYENQKLIANQFNSAIGKIQDSLSSTASALGKLQDVVNQNAQALNTLVKQLSSNFGAISSVLNDILSRLDKVEAEVQIDRLITGRLQSLQTYVTQQLIRAAEIRASANLAATKMSECVLGQSKRVDFCGKGYHLMSFPQSAPHGVVFLHVTYVPAQEKNFTTAPAICHDGKAHFPREGVFVSNGTHWFVTQRNFYEPQIITTDNTFVSGNCDVVIGIVNNTVYDPLQPELDSFKEELDKYFKNHTSPDVDLGDISGINASVVNIQKEIDRLNEVAKNLNESLIDLQELGKYEQYIKWPWYIWLGFIAGLIAIVMVTIMLCCMTSCCSCLKGCCSCGSCCKFDEDDSEPVLKGVKLHYT

SEQ ID NO: 2 - protein, 1273 aa, Artificial Sequence
  full-length S protein fixed in the pre-fusion conformation
MFVFLVLLPLVSSQCVNLTTRTQLPPAYTNSFTRGVYYPDKVFRSSVLHSTQDLFLPFFSNVTWFHAIHVSGTNGTKRFDNPVLPFNDGVYFASTEKSNIIRGWIFGTTLDSKTQSLLIVNNATNVVIKVCEFQFCNDPFLGVYYHKNNKSWMESEFRVYSSANNCTFEYVSQPFLMDLEGKQGNFKNLREFVFKNIDGYFKIYSKHTPINLVRDLPQGFSALEPLVDLPIGINITRFQTLLALHRSYLTPGDSSSGWTAGAAAYYVGYLQPRTFLLKYNENGTITDAVDCALDPLSETKCTLKSFTVEKGIYQTSNFRVQPTESIVRFPNITNLCPFGEVFNATRFASVYAWNRKRISNCVADYSVLYNSASFSTFKCYGVSPTKLNDLCFTNVYADSFVIRGDEVRQIAPGQTGKIADYNYKLPDDFTGCVIAWNSNNLDSKVGGNYNYLYRLFRKSNLKPFERDISTEIYQAGSTPCNGVEGFNCYFPLQSYGFQPTNGVGYQPYRVVVLSFELLHAPATVCGPKKSTNLVKNKCVNFNFNGLTGTGVLTESNKKFLPFQQFGRDIADTTDAVRDPQTLEILDITPCSFGGVSVITPGTNTSNQVAVLYQDVNCTEVPVAIHADQLTPTWRVYSTGSNVFQTRAGCLIGAEHVNNSYECDIPIGAGICASYQTQTNSPGSAGSVASQSIIAYTMSLGAENSVAYSNNSIAIPTNFTISVTTEILPVSMTKTSVDCTMYICGDSTECSNLLLQYGSFCTQLNRALTGIAVEQDKNTQEVFAQVKQIYKTPPIKDFGGFNFSQILPDPSKPSKRSFIEDLLFNKVTLADAGFIKQYGDCLGDIAARDLICAQKFNGLTVLPPLLTDEMIAQYTSALLAGTITSGWTFGAGAALQIPFAMQMAYRFNGIGVTQNVLYENQKLIANQFNSAIGKIQDSLSSTASALGKLQDVVNQNAQALNTLVKQLSSNFGAISSVLNDILSRLDPPEAEVQIDRLITGRLQSLQTYVTQQLIRAAEIRASANLAATKMSECVLGQSKRVDFCGKGYHLMSFPQSAPHGVVFLHVTYVPAQEKNFTTAPAICHDGKAHFPREGVFVSNGTHWFVTQRNFYEPQIITTDNTFVSGNCDVVIGIVNNTVYDPLQPELDSFKEELDKYFKNHTSPDVDLGDISGINASVVNIQKEIDRLNEVAKNLNESLIDLQELGKYEQYIKWPWYIWLGFIAGLIAIVMVTIMLCCMTSCCSCLKGCCSCGSCCKFDEDDSEPVLKGVKLHYT

SEQ ID NO: 3 - protein, 198 aa, Artificial Sequence
  RBD
ITNLCPFGEVFNATRFASVYAWNRKRISNCVADYSVLYNSASFSTFKCYGVSPTKLNDLCFTNVYADSFVIRGDEVRQIAPGQTGKIADYNYKLPDDFTGCVIAWNSNNLDSKVGGNYNYLYRLFRKSNLKPFERDISTEIYQAGSTPCNGVEGFNCYFPLQSYGFQPTNGVGYQPYRVVVLSFELLHAPATVCGPKK

SEQ ID NO: 4 - DNA, 666 bp, Artificial Sequence
  Nucleotide sequence encoding wild-type SARS-CoV-2 RBD with tPA signal peptide
atggacgccatgaagaggggactgtgctgcgtgctgctgctgtgcggagccgtgttcgtgagcaactccatcaccaacctgtgccccttcggcgaggtgtttaacgccacacgctttgcctccgtgtatgcctggaaccggaagagaatctccaattgcgtggccgactattctgtgctgtacaattctgccagcttctccacctttaagtgctatggcgtgtctcctaccaagctgaacgacctgtgcttcacaaacgtgtacgccgacagctttgtgatccggggcgatgaggtgagacagatcgcaccaggacagaccggcaagatcgcagactacaactataagctgcccgacgatttcacaggctgcgtgatcgcctggaattctaacaatctggatagcaaagtgggcggcaactacaattatctgtacaggctgttccgcaagagcaacctgaagccttttgagcgggacatcagcaccgagatctaccaggccggctccacaccatgcaacggcgtggagggcttcaattgttattttccactgcagtcctacggcttccagcccaccaatggcgtgggctatcagccttaccgggtggtggtgctgtcttttgagctgctgcacgcaccagcaacagtgtgcggacctaagaagtga

SEQ ID NO: 5 - DNA, 3786 bp, Artificial Sequence
  Nucleotide sequence encoding full-length S protein fixed in the pre-fusion conformation with a mutation to GSAG at 682RRAR685 and a mutation to PP at 986KV987
tcccagtgcgtgaacctgaccacaaggacccagctgccacctgcctataccaatagcttcacaagaggcgtgtactatcctgacaaggtgtttcgctctagcgtgctgcactctacacaggatctgtttctgccattctttagcaacgtgacctggttccacgccatccacgtgtccggcaccaatggcacaaagagattcgacaatccagtgctgccctttaacgatggcgtgtacttcgctagcaccgagaagtccaacatcatccgcggctggatctttggcaccacactggactctaagacacagagcctgctgatcgtgaacaatgccaccaacgtggtcatcaaggtgtgcgagttccagttttgtaatgatcccttcctgggcgtgtactatcacaagaacaataagtcctggatggagtctgagtttagggtgtattcctctgccaacaattgcacatttgagtacgtgtcccagcctttcctgatggacctggagggcaagcagggcaatttcaagaacctgcgggagttcgtgtttaagaatatcgatggctacttcaagatctactccaagcacacccctatcaacctggtgagggacctgccacagggcttctctgccctggagcctctggtggatctgccaatcggcatcaacatcaccagatttcagacactgctggctctgcaccgcagctacctgacacccggcgacagctcctctggatggaccgctggagctgctgcttactatgtgggctatctgcagcctcggaccttcctgctgaagtacaacgagaatggcaccatcacagacgctgtggattgcgccctggatcctctgagcgagaccaagtgtacactgaagtcctttaccgtggagaagggcatctatcagacatccaatttccgggtgcagccaaccgagtctatcgtgaggtttccaaatatcacaaacctgtgcccctttggcgaggtgttcaacgctaccaggttcgccagcgtgtacgcttggaatagaaagcgcatctctaactgcgtggctgactatagcgtgctgtacaacagcgcctccttctctacctttaagtgctatggcgtgagccctacaaagctgaatgacctgtgctttaccaacgtgtacgccgattccttcgtgatcagaggcgacgaggtgcgccagatcgctccaggacagacaggcaagatcgccgactacaattataagctgcccgacgatttcaccggctgcgtgatcgcctggaactccaacaatctggattctaaagtgggcggcaactacaattatctgtaccggctgtttaggaagtccaatctgaagcccttcgagcgggacatctctacagagatctaccaggccggcagcaccccttgcaatggcgtggagggctttaactgttatttccccctgcagtcttacggcttccagcctacaaacggcgtgggctatcagccatacagggtggtggtgctgtcttttgagctgctgcacgctccagctacagtgtgcggacctaagaagagcaccaatctggtgaagaacaagtgcgtgaacttcaacttcaacggactgaccggaacaggcgtgctgaccgagtctaacaagaagttcctgccatttcagcagttcggccgggacatcgccgataccacagacgctgtgagggacccccagaccctggagatcctggatatcacaccttgcagcttcggcggcgtgtccgtgatcacaccaggaaccaatacaagcaaccaggtggccgtgctgtatcaggacgtgaattgtaccgaggtgccagtggctatccacgccgatcagctgacccccacatggagagtgtactctaccggcagcaacgtgtttcagacaagggctggatgtctgatcggagctgagcacgtgaacaatagctatgagtgcgacatcccaatcggcgccggcatctgtgcttcctaccagacccagacaaactctccaggctccgccggcagcgtggctagccagtccatcatcgcttataccatgtccctgggcgccgagaattctgtggcttactccaacaattctatcgccatccccaccaacttcacaatcagcgtgaccacagagatcctgcccgtgagcatgaccaagacaagcgtggactgcacaatgtatatctgtggcgatagcaccgagtgctccaacctgctgctgcagtacggctccttttgtacccagctgaatcgcgccctgacaggcatcgctgtggagcaggataagaacacacaggaggtgttcgcccaggtgaagcagatctacaagaccccacccatcaaggactttggcggcttcaatttttcccagatcctgcccgatcctagcaagccttccaagagatcttttatcgaggacctgctgttcaacaaggtgaccctggctgatgccggcttcatcaagcagtatggcgattgcctgggcgacatcgctgctagggacctgatctgtgctcagaagtttaatggcctgaccgtgctgcctccactgctgacagatgagatgatcgctcagtacacaagcgccctgctggctggaaccatcacatccggatggaccttcggcgctggagctgccctgcagatcccatttgccatgcagatggcttatagattcaacggcatcggcgtgacccagaatgtgctgtacgagaaccagaagctgatcgccaatcagtttaactccgctatcggcaagatccaggacagcctgagcagcacagcttccgccctgggcaagctgcaggatgtggtgaatcagaacgctcaggccctgaataccctggtgaagcagctgtctagcaacttcggcgctatctcctctgtgctgaatgatatcctgagccggctggaccctccagaggctgaggtgcagatcgaccggctgatcacaggcaggctgcagtccctgcagacctatgtgacacagcagctgatcagagctgccgagatccgcgcttctgccaatctggctgccaccaagatgtccgagtgcgtgctgggccagtctaagcgcgtggacttttgtggcaagggctatcacctgatgtctttcccacagagcgccccacacggagtggtgtttctgcacgtgacctacgtgcctgcccaggagaagaacttcaccacagctccagccatctgccacgatggcaaggcccactttccacgggagggcgtgttcgtgagcaacggcacccactggtttgtgacacagaggaatttctacgagccccagatcatcaccacagacaataccttcgtgagcggcaactgtgacgtggtcatcggcatcgtgaacaataccgtgtatgatcctctgcagccagagctggactcttttaaggaggagctggataagtacttcaagaatcacaccagccccgacgtggatctgggcgacatctccggcatcaatgcttctgtggtgaacatccagaaggagatcgaccgcctgaacgaggtggccaagaatctgaacgagagcctgatcgatctgcaggagctgggcaagtatgagcagtacatcaagtggccctggtatatctggctgggcttcatcgccggcctgatcgccatcgtgatggtgaccatcatgctgtgctgtatgacaagctgctgttcctgcctgaagggctgctgttcttgtggcagctgctgtaagtttgatgaggacgatagcgagcctgtgctgaagggcgtgaagctgcactacacctga

SEQ ID NO: 6 - DNA, 3786 bp, Artificial Sequence
  nucleotide sequence encoding a wild-type 2019-nCoV S protein without signal peptide
tcccagtgcgtgaacctgaccacaaggacccagctgccccctgcctataccaattccttcacacggggcgtgtactatcccgacaaggtgtttagatctagcgtgctgcactccacacaggatctgtttctgcctttcttttctaacgtgacctggttccacgccatccacgtgagcggcaccaatggcacaaagcggttcgacaatccagtgctgccctttaacgatggcgtgtacttcgcctccaccgagaagtctaacatcatcagaggctggatctttggcaccacactggacagcaagacacagtccctgctgatcgtgaacaatgccaccaacgtggtcatcaaggtgtgcgagttccagttttgtaatgatccattcctgggcgtgtactatcacaagaacaataagtcttggatggagagcgagtttcgcgtgtattcctctgccaacaattgcacatttgagtacgtgtcccagcccttcctgatggacctggagggcaagcagggcaatttcaagaacctgagggagttcgtgtttaagaatatcgatggctacttcaagatctactccaagcacaccccaatcaacctggtgcgcgacctgccacagggcttctctgccctggagccactggtggatctgcccatcggcatcaacatcacccggtttcagacactgctggccctgcacagaagctacctgacaccaggcgacagctcctctggatggaccgcaggagcagcagcctactatgtgggctatctgcagcccaggaccttcctgctgaagtacaacgagaatggcaccatcacagacgccgtggattgcgccctggatcccctgtctgagaccaagtgtacactgaagagctttaccgtggagaagggcatctatcagacaagcaatttcagggtgcagcctaccgagtccatcgtgcgctttcccaatatcacaaacctgtgcccttttggcgaggtgttcaacgcaaccaggttcgcaagcgtgtacgcatggaataggaagcgcatctccaactgcgtggccgactattctgtgctgtacaacagcgcctccttctctacctttaagtgctatggcgtgagccccacaaagctgaatgacctgtgctttaccaacgtgtacgccgattccttcgtgatcaggggcgacgaggtgcgccagatcgcaccaggacagacaggcaagatcgcagactacaattataagctgcctgacgatttcaccggctgcgtgatcgcctggaactctaacaatctggatagcaaagtgggcggcaactacaattatctgtaccggctgtttagaaagtctaatctgaagccattcgagagggacatctccacagagatctaccaggccggctctaccccctgcaatggcgtggagggctttaactgttatttccctctgcagagctacggcttccagccaacaaacggcgtgggctatcagccctaccgcgtggtggtgctgtcttttgagctgctgcacgcacctgcaacagtgtgcggaccaaagaagagcaccaatctggtgaagaacaagtgcgtgaacttcaacttcaacggactgaccggaacaggcgtgctgaccgagtccaacaagaagttcctgccttttcagcagttcggcagggacatcgcagataccacagacgccgtgcgcgaccctcagaccctggagatcctggacatcacaccatgctccttcggcggcgtgtctgtgatcacaccaggcaccaatacaagcaaccaggtggccgtgctgtatcaggacgtgaattgtaccgaggtgccagtggcaatccacgcagatcagctgacccctacatggcgggtgtactctaccggcagcaacgtgttccagacaagagcaggatgcctgatcggagcagagcacgtgaacaatagctatgagtgcgacatccctatcggcgccggcatctgtgcctcctaccagacccagacaaactccccaaggagagcacggtctgtggcaagccagtccatcatcgcctataccatgagcctgggcgccgagaattccgtggcctactccaacaattctatcgccatccctaccaacttcacaatctccgtgaccacagagatcctgccagtgagcatgaccaagacatccgtggactgcacaatgtatatctgtggcgattccaccgagtgctctaacctgctgctgcagtacggctctttttgtacccagctgaatagagccctgacaggcatcgccgtggagcaggacaagaacacacaggaggtgttcgcccaggtgaagcagatctacaagaccccacccatcaaggactttggcggcttcaacttcagccagatcctgcccgatcctagcaagccatccaagcggtcttttatcgaggacctgctgttcaacaaggtgaccctggccgatgccggcttcatcaagcagtatggcgattgcctgggcgacatcgccgccagagacctgatctgtgcccagaagtttaatggcctgaccgtgctgcctccactgctgacagatgagatgatcgcccagtacacatctgccctgctggcaggaaccatcacaagcggatggaccttcggcgcaggagccgccctgcagatcccctttgccatgcagatggcctatcggttcaacggcatcggcgtgacccagaatgtgctgtacgagaaccagaagctgatcgccaatcagtttaactccgccatcggcaagatccaggactctctgagctccacagcaagcgccctgggcaagctgcaggatgtggtgaatcagaacgcccaggccctgaataccctggtgaagcagctgtctagcaacttcggcgccatctcctctgtgctgaatgacatcctgagcaggctggacaaggtggaggcagaggtgcagatcgaccggctgatcacaggcagactgcagtccctgcagacctacgtgacacagcagctgatcagggcagcagagatcagggcatctgccaatctggccgccaccaagatgagcgagtgcgtgctgggccagtccaagagagtggacttttgtggcaagggctatcacctgatgagcttcccacagtccgcccctcacggagtggtgtttctgcacgtgacctacgtgccagcccaggagaagaacttcaccacagcaccagcaatctgccacgatggcaaggcacactttcctagggagggcgtgttcgtgagcaacggcacccactggtttgtgacacagcgcaatttctacgagccacagatcatcaccacagacaatacattcgtgtccggcaactgtgacgtggtcatcggcatcgtgaacaataccgtgtatgatcctctgcagccagagctggactcttttaaggaggagctggataagtacttcaagaatcacaccagccccgacgtggatctgggcgacatctctggcatcaatgccagcgtggtgaacatccagaaggagatcgacaggctgaacgaggtggccaagaatctgaacgagtccctgatcgatctgcaggagctgggcaagtatgagcagtacatcaagtggccctggtatatctggctgggcttcatcgccggcctgatcgccatcgtgatggtgaccatcatgctgtgctgtatgacaagctgctgttcctgcctgaagggctgctgttcttgtggcagctgctgtaagtttgatgaggacgatagcgagcctgtgctgaagggcgtgaagctgcactacacctga

SEQ ID NO: 7 - DNA, 651 bp, Artificial Sequence
  Nucleotide sequence encoding the RBD of wild-type SARS-CoV-2 containing IgE signal peptide
atggattggacgtggatcttgttcctggtggcggcggccaccagggtacattccatcaccaatctatgcccgtttggcgaggtgttcaacgccacgcgatttgcctcagtttacgcctggaatcgcaagcgaatcagcaattgcgtcgcagattattcagttttgtacaactcggcatcctttagcacgttcaagtgctatggggtgtcgcccacaaaactgaatgatctgtgtttcaccaacgtatatgctgattcgtttgtgattcggggcgatgaagtgaggcagatcgcgcctggccagacgggcaagatcgccgactacaactacaagttgccggacgattttacaggctgtgtgattgcgtggaacagtaacaacctcgactccaaggtagggggtaactacaactacctgtatagactctttcgaaagtccaacttgaagccattcgagcgggacatttcgacagagatctatcaggcaggtagtaccccctgcaatggagtcgagggcttcaattgttactttccactgcagtcatacggcttccaacctactaatggggtcgggtaccagccgtaccgcgtggtggtgctcagctttgagctcctccacgcgccggctacggtatgcggccccaagaagtag

SEQ ID NO: 8 - DNA, 319 bp, Artificial Sequence
  A base plasmid template comprising T7 promoter, 5' UTR, 3' UTR and polyA tail
  misc_feature (308)..(312): n is a, c, g, t or u
taatacgactcactatagggaaataagagagaaaagaagagtaagaagaaatataagagccaccggagacggattgattgccgtctcctgataataggctggagcctcggtggccatgcttcttgccccttgggcctccccccagcccctcctccccttcctgcacccgtacccccgtggtctttgaataaagtctgagtgggcggcaaaaaaaaaaaaaaaaaaaaaaaaaaaaaaaaaaaaaaaaaaaaaaaaaaaaaaaaaaaaaaaaaaaaaaaaaaaaaaaaaaaaaaaaaaaaaaaaaaaannnnnggtcttc

SEQ ID NO: 9 - DNA, 651 bp, Artificial Sequence)
  Nucleotide sequence encoding the RBD of wild-type SARS-CoV-2 containing IgE signal peptide
atggactggacctggatcctcttcctcgtggccgccgccacccgcgtgcacagcatcaccaacctgtgccccttcggcgaggtgtttaacgccacacgctttgcctccgtgtatgcctggaaccggaagagaatctccaattgcgtggccgactattctgtgctgtacaattctgccagcttctccacctttaagtgctatggcgtgtctcctaccaagctgaacgacctgtgcttcacaaacgtgtacgccgacagctttgtgatccggggcgatgaggtgagacagatcgcaccaggacagaccggcaagatcgcagactacaactataagctgcccgacgatttcacaggctgcgtgatcgcctggaattctaacaatctggatagcaaagtgggcggcaactacaattatctgtacaggctgttccgcaagagcaacctgaagccttttgagcgggacatcagcaccgagatctaccaggccggctccacaccatgcaacggcgtggagggcttcaattgttattttccactgcagtcctacggcttccagcccaccaatggcgtgggctatcagccttaccgggtggtggtgctgtcttttgagctgctgcacgcaccagcaacagtgtgcggacctaagaagtga

SEQ ID NO: 10 - DNA, 651 bp, Artificial Sequence
  Nucleotide sequence encoding the RBD of wild-type SARS-CoV-2 containing IgE signal peptide
atggactggacctggatcctcttcctcgtggccgccgccacccgggtgcacagcatcaccaacctctgccccttcggggaggtcttcaacgccacccgcttcgccagcgtctacgcctggaaccgcaagcgcatctccaactgcgtggccgactacagcgtgctgtacaacagcgcctccttctccaccttcaagtgctacggggtcagccccaccaagctgaacgacctctgcttcaccaacgtctacgcggactccttcgtcatccggggggacgaggtgcggcagatcgccccgggccagacgggcaagatcgccgactacaactacaagctgccggacgacttcacgggctgcgtcatcgcctggaacagcaacaacctggacagcaaggtgggcggcaactacaactacctgtaccgcctcttccgcaagtccaacctgaagcccttcgagcgggacatctccacggagatctaccaggcgggctccaccccctgcaacggggtggagggcttcaactgctacttccccctgcagagctacggcttccagcccaccaacggggtgggctaccagccctaccgggtggtggtgctgtccttcgagctgctgcacgcgccggccaccgtgtgcgggcccaagaagtga

SEQ ID NO: 11 - DNA, 651 bp, Artificial Sequence
  Nucleotide sequence encoding the RBD of wild-type SARS-CoV-2 containing IgE signal peptide
atggactggacctggatcctcttcctggtggccgccgccacccgggtgcacagcatcaccaacctctgccccttcggggaggtcttcaacgccacccgcttcgccagcgtctacgcctggaaccgcaagcgcatctccaactgcgtggccgactacagcgtgctgtacaacagcgcctccttctccaccttcaagtgctacggggtcagccccaccaagctgaacgacctctgcttcaccaacgtctacgcggactccttcgtcatccggggggacgaggtgcggcagatcgccccgggccagacgggcaagatcgccgactacaactacaagctgccggacgacttcacgggctgcgtcatcgcctggaacagcaacaacctggacagcaaggtgggcggcaactacaactacctctaccgcctcttccgcaagtccaacctgaagcccttcgagcgggacatctccacggagatctaccaggcgggctccaccccctgcaacggggtggagggcttcaactgctacttccccctgcagagctacggcttccagcccaccaacggggtgggctaccagccctaccgggtggtggtgctgtccttcgagctgctgcacgcgccggccaccgtgtgcgggcccaagaagtga

SEQ ID NO: 12 - DNA, 726 bp, Artificial Sequence
  Nucleotide sequence encoding RBD of wild type SARS CoV-2 containing IgE signal peptide, including K417N, E484K and N501Y mutations of 501Y.V2 family
atggactggacctggatcctgttcctggtcgccgctgccacccgggtgcacagcagagtgcagcccaccgagtctatcgtgcggtttcccaacatcaccaacctctgtcctttcggcgaagtctttaacgccacaagattcgccagcgtttacgcctggaataggaaaagaatcagcaattgcgtggccgactacagcgtgctgtacaacagcgcctctttcagcaccttcaagtgttacggagtgtcccctacaaagctgaacgacctgtgcttcacaaacgtgtacgctgattcttttgtgattagaggcgacgaggtgcggcagatcgcccctggccagaccggcaacatcgctgattacaactataagctgcctgacgacttcaccggatgtgtgatcgcctggaacagcaataacctggactccaaggtgggaggcaattacaactacctgtaccggctgttcagaaagtccaacctgaagcccttcgaaagagatatcagcacagagatctaccaggccggcagcaccccatgcaacggcgtgaagggcttcaactgctacttccccctgcagagctacggctttcagcctacctacggcgtgggttatcaaccatacagagtggtggtcctgagcttcgagctgctgcacgcccctgccaccgtgtgcggccctaagaaatctacaaatctggtgaaaaacaagtgcgtgaacttctaa

SEQ ID NO: 13 - protein, 241 aa, Artificial Sequence
  RBD
MDWTWILFLVAAATRVHSRVQPTESIVRFPNITNLCPFGEVFNATRFASVYAWNRKRISNCVADYSVLYNSASFSTFKCYGVSPTKLNDLCFTNVYADSFVIRGDEVRQIAPGQTGNIADYNYKLPDDFTGCVIAWNSNNLDSKVGGNYNYLYRLFRKSNLKPFERDISTEIYQAGSTPCNGVKGFNCYFPLQSYGFQPTYGVGYQPYRVVVLSFELLHAPATVCGPKKSTNLVKNKCVNF

SEQ ID NO: 14 - DNA, 3813 bp, Artificial Sequence
  The nucleotide sequence encoding the mutant S protein
atgttcgtgtttctggtgctgctgcccctggtgagctcccagtgcgtgaatttcaccaccagaacccagctgccacctgcctataccaacagtttcaccagaggcgtgtactaccccgataaggtgtttagatccagcgtgctgcacagcacccaagacctgtttctgcccttcttcagcaacgtgacctggttccacgctatccacgtgagcggcaccaacggcactaagaggttcgccaatcctgtgctgcctttcaacgacggcgtatattttgccagcaccgaaaagagcaacatcatcagaggatggatcttcggaaccaccctggacagcaagacccagagcctgctgatcgtgaacaacgccaccaacgtggtgatcaaggtgtgtgaattccaattctgcaacgaccctttcctgggagtctactaccacaagaacaacaagagctggatggaatccgagttcagagtgtactctagcgctaataactgcacctttgagtacgtgagccagccattcctgatggacctggaaggcaagcaaggcaacttcaagaatttgcgggaattcgtcttcaaaaacatcgacggctacttcaagatctacagcaagcacacccccatcaacctggtcagaggactgcctcaaggcttttctgctctggaacctctagttgacctgcctatcggcattaacatcacaagattccagacactgcacatcagctacctgacccctggagatagctctagcggatggacagccggcgctgccgcctactacgtgggatatctgcagcccagaacattcctgctgaaatacaacgagaacggtacaatcaccgacgccgtggactgcgccctggaccctctgtctgagacaaagtgcacgctgaagtccttcacagtggaaaagggcatctatcagaccagcaatttccgcgtgcagcctaccgagagcatagtgcggttccccaacatcaccaacctgtgtccttttggcgaggtgttcaatgccacacggttcgcctccgtgtacgcctggaacagaaagcggatcagcaattgcgtggccgactactccgtgctgtacaacagcgccagcttcagcaccttcaagtgctacggcgtgtcccctacgaaactgaacgatctgtgcttcaccaacgtgtacgccgacagcttcgtgatccgaggcgacgaggtgagacagatcgcccctggccagaccggcaacatcgccgattacaactacaagctgcctgacgacttcaccggctgcgtgatcgcctggaatagcaacaacctggattctaaagtgggcggcaattacaactacctgtacagactgttcagaaagtcgaacctgaaacctttcgagagagatatctctaccgagatctaccaggccggcagcaccccctgcaatggcgtcaaaggcttcaactgttacttccctctgcagagctacggctttcagccaacctacggcgtcggctaccagccatacagagtggtagtgctcagcttcgagctgctgcatgcccccgccacagtttgtggccctaagaaaagcacaaatctggtgaagaacaagtgcgtgaacttcaacttcaacggcctgacaggcaccggagtgctcaccgagagcaacaaaaagttcctgcctttccagcagtttgggagagatatcgcagacaccacagatgccgtgcgggacccccagaccctcgaaatcctggacatcacaccttgtagctttggaggcgtgtctgtgattacacctggcacaaacacaagcaaccaggtggctgtgctgtaccaaggcgtcaactgcaccgaagtgcccgtggctatccacgccgaccagctgaccccgacctggcgggtgtacagcacaggcagtaatgtgtttcagacccgggccggctgtctgatcggagccgagcacgtgaacaacagctacgagtgcgacatccccatcggcgccggcatctgcgcctcttatcagacacagacaaacagccccggatctgctggcagcgttgctagccagtctatcattgcctacaccatgtccctgggcgtggagaattctgtggcttactccaacaattctatcgccatccccaccaacttcacaatcagcgtgaccacagagatcctgcccgtgagcatgaccaagacaagcgtggactgcacaatgtatatctgtggcgacagcaccgagtgctccaacctgctgctgcagtacggctccttttgtacccagctgaatcgcgccctgacaggcatcgctgtggagcaggacaagaacacacaggaggtgttcgcccaggtgaagcagatctacaagaccccacccatcaaggactttggcggcttcaatttttcccagatcctgcccgatcccagcaagccttccaagagatcttttatcgaggacctgctgttcaacaaggtgaccctggccgatgccggcttcatcaagcagtatggcgattgcctgggcgacatcgctgccagggacctgatctgtgctcagaagttcaatggcctgaccgtgctgcctccactgctgacagacgagatgatcgctcagtacacaagcgccctgctggctggaaccatcacatccggctggaccttcggcgctggagctgccctgcagatcccatttgccatgcagatggcttacagattcaacggcatcggcgtgacccagaatgtgctgtacgagaaccagaagctgatcgccaatcagttcaactccgctatcggcaagatccaggacagcctgagcagcacagcttccgccctgggcaagctgcaggatgtggtgaatcagaacgctcaggccctgaataccctggtgaagcagctgtcgagcaacttcggcgctatctcctctgtgctgaacgatatcctgagccggctggaccctccagaggcggaggtgcagatcgaccggctgatcacaggcaggctgcagtccctgcagacctatgtgacacagcagctgatcagagctgccgagatccgcgcttctgccaatctggctgccaccaagatgtccgagtgcgtgctgggccagtcgaagcgcgtggacttttgtggcaagggctatcacctgatgtctttcccacagagcgccccacacggagtggtgtttctgcacgtgacctacgtgcctgcccaggagaagaacttcaccacagctccagccatctgccacgatggcaaggcccactttccacgggagggcgtgttcgtgagcaacggcacccactggtttgtgacacagaggaatttctacgagccccagatcatcaccacagacaataccttcgtgagcggcaactgcgacgtggtcatcggcatcgtgaacaataccgtgtacgatcctctgcagccagagctggactctttcaaggaggagctggacaagtacttcaagaatcacaccagccccgacgtggatctgggcgacatctccggcatcaatgcttctgtggtgaacatccagaaggagatcgaccgcctgaacgaggtggccaagaatctgaacgagagcctgatcgatctgcaggagctgggcaagtacgagcagtacatcaagtggccctggtatatctggctgggcttcatcgccggcctgatcgccatcgtgatggtgaccatcatgctgtgctgtatgacaagctgctgttcctgcctgaagggctgctgttcttgtggcagctgctgcaagttcgacgaggacgacagcgagcctgtgctgaagggcgtgaagctgcactacacctaa

SEQ ID NO: 15 - protein, 1270 aa, Artificial Sequence
  full-length S protein fixed in the pre-fusion conformation
MFVFLVLLPLVSSQCVNFTTRTQLPPAYTNSFTRGVYYPDKVFRSSVLHSTQDLFLPFFSNVTWFHAIHVSGTNGTKRFANPVLPFNDGVYFASTEKSNIIRGWIFGTTLDSKTQSLLIVNNATNVVIKVCEFQFCNDPFLGVYYHKNNKSWMESEFRVYSSANNCTFEYVSQPFLMDLEGKQGNFKNLREFVFKNIDGYFKIYSKHTPINLVRGLPQGFSALEPLVDLPIGINITRFQTLHISYLTPGDSSSGWTAGAAAYYVGYLQPRTFLLKYNENGTITDAVDCALDPLSETKCTLKSFTVEKGIYQTSNFRVQPTESIVRFPNITNLCPFGEVFNATRFASVYAWNRKRISNCVADYSVLYNSASFSTFKCYGVSPTKLNDLCFTNVYADSFVIRGDEVRQIAPGQTGNIADYNYKLPDDFTGCVIAWNSNNLDSKVGGNYNYLYRLFRKSNLKPFERDISTEIYQAGSTPCNGVKGFNCYFPLQSYGFQPTYGVGYQPYRVVVLSFELLHAPATVCGPKKSTNLVKNKCVNFNFNGLTGTGVLTESNKKFLPFQQFGRDIADTTDAVRDPQTLEILDITPCSFGGVSVITPGTNTSNQVAVLYQGVNCTEVPVAIHADQLTPTWRVYSTGSNVFQTRAGCLIGAEHVNNSYECDIPIGAGICASYQTQTNSPGSAGSVASQSIIAYTMSLGVENSVAYSNNSIAIPTNFTISVTTEILPVSMTKTSVDCTMYICGDSTECSNLLLQYGSFCTQLNRALTGIAVEQDKNTQEVFAQVKQIYKTPPIKDFGGFNFSQILPDPSKPSKRSFIEDLLFNKVTLADAGFIKQYGDCLGDIAARDLICAQKFNGLTVLPPLLTDEMIAQYTSALLAGTITSGWTFGAGAALQIPFAMQMAYRFNGIGVTQNVLYENQKLIANQFNSAIGKIQDSLSSTASALGKLQDVVNQNAQALNTLVKQLSSNFGAISSVLNDILSRLDPPEAEVQIDRLITGRLQSLQTYVTQQLIRAAEIRASANLAATKMSECVLGQSKRVDFCGKGYHLMSFPQSAPHGVVFLHVTYVPAQEKNFTTAPAICHDGKAHFPREGVFVSNGTHWFVTQRNFYEPQIITTDNTFVSGNCDVVIGIVNNTVYDPLQPELDSFKEELDKYFKNHTSPDVDLGDISGINASVVNIQKEIDRLNEVAKNLNESLIDLQELGKYEQYIKWPWYIWLGFIAGLIAIVMVTIMLCCMTSCCSCLKGCCSCGSCCKFDEDDSEPVLKGVKLHYT

SEQ ID NO: 16 - RNA, 930 nt, Artificial Sequence
  mRNA
ggggaaauaagagagaaaagaagaguaagaagaaauauaagagccaccauggacgccaugaagaggggacugugcugcgugcugcugcugugcggagccguguucgugagcaacuccaucaccaaccugugccccuucggcgagguguuuaacgccacacgcuuugccuccguguaugccuggaaccggaagagaaucuccaauugcguggccgacuauucugugcuguacaauucugccagcuucuccaccuuuaagugcuauggcgugucuccuaccaagcugaacgaccugugcuucacaaacguguacgccgacagcuuugugauccggggcgaugaggugagacagaucgcaccaggacagaccggcaagaucgcagacuacaacuauaagcugcccgacgauuucacaggcugcgugaucgccuggaauucuaacaaucuggauagcaaagugggcggcaacuacaauuaucuguacaggcuguuccgcaagagcaaccugaagccuuuugagcgggacaucagcaccgagaucuaccaggccggcuccacaccaugcaacggcguggagggcuucaauuguuauuuuccacugcaguccuacggcuuccagcccaccaauggcgugggcuaucagccuuaccgggugguggugcugucuuuugagcugcugcacgcaccagcaacagugugcggaccuaagaagugauaauaggcuggagccucgguggccaugcuucuugccccuugggccuccccccagccccuccuccccuuccugcacccguacccccguggucuuugaauaaagucugagugggcggcaaaaaaaaaaaaaaaaaaaaaaaaaaaaaaaaaaaaaaaaaaaaaaaaaaaaaaaaaaaaaaaaaaaaaaaaaaaaaaaaaaaaaaaaaaaaaaaaaaaa

SEQ ID NO: 17 - RNA, 4086 nt, Artificial Sequence
  mRNA
ggggaaauaagagagaaaagaagaguaagaagaaauauaagagccaccauguucguguuucuggugcugcugccccuggugagcucccagugcgugaaccugaccacaaggacccagcugccaccugccuauaccaauagcuucacaagaggcguguacuauccugacaagguguuucgcucuagcgugcugcacucuacacaggaucuguuucugccauucuuuagcaacgugaccugguuccacgccauccacguguccggcaccaauggcacaaagagauucgacaauccagugcugcccuuuaacgauggcguguacuucgcuagcaccgagaaguccaacaucauccgcggcuggaucuuuggcaccacacuggacucuaagacacagagccugcugaucgugaacaaugccaccaacguggucaucaaggugugcgaguuccaguuuuguaaugaucccuuccugggcguguacuaucacaagaacaauaaguccuggauggagucugaguuuaggguguauuccucugccaacaauugcacauuugaguacgugucccagccuuuccugauggaccuggagggcaagcagggcaauuucaagaaccugcgggaguucguguuuaagaauaucgauggcuacuucaagaucuacuccaagcacaccccuaucaaccuggugagggaccugccacagggcuucucugcccuggagccucugguggaucugccaaucggcaucaacaucaccagauuucagacacugcuggcucugcaccgcagcuaccugacacccggcgacagcuccucuggauggaccgcuggagcugcugcuuacuaugugggcuaucugcagccucggaccuuccugcugaaguacaacgagaauggcaccaucacagacgcuguggauugcgcccuggauccucugagcgagaccaaguguacacugaaguccuuuaccguggagaagggcaucuaucagacauccaauuuccgggugcagccaaccgagucuaucgugagguuuccaaauaucacaaaccugugccccuuuggcgagguguucaacgcuaccagguucgccagcguguacgcuuggaauagaaagcgcaucucuaacugcguggcugacuauagcgugcuguacaacagcgccuccuucucuaccuuuaagugcuauggcgugagcccuacaaagcugaaugaccugugcuuuaccaacguguacgccgauuccuucgugaucagaggcgacgaggugcgccagaucgcuccaggacagacaggcaagaucgccgacuacaauuauaagcugcccgacgauuucaccggcugcgugaucgccuggaacuccaacaaucuggauucuaaagugggcggcaacuacaauuaucuguaccggcuguuuaggaaguccaaucugaagcccuucgagcgggacaucucuacagagaucuaccaggccggcagcaccccuugcaauggcguggagggcuuuaacuguuauuucccccugcagucuuacggcuuccagccuacaaacggcgugggcuaucagccauacagggugguggugcugucuuuugagcugcugcacgcuccagcuacagugugcggaccuaagaagagcaccaaucuggugaagaacaagugcgugaacuucaacuucaacggacugaccggaacaggcgugcugaccgagucuaacaagaaguuccugccauuucagcaguucggccgggacaucgccgauaccacagacgcugugagggacccccagacccuggagauccuggauaucacaccuugcagcuucggcggcguguccgugaucacaccaggaaccaauacaagcaaccagguggccgugcuguaucaggacgugaauuguaccgaggugccaguggcuauccacgccgaucagcugacccccacauggagaguguacucuaccggcagcaacguguuucagacaagggcuggaugucugaucggagcugagcacgugaacaauagcuaugagugcgacaucccaaucggcgccggcaucugugcuuccuaccagacccagacaaacucuccaggcuccgccggcagcguggcuagccaguccaucaucgcuuauaccaugucccugggcgccgagaauucuguggcuuacuccaacaauucuaucgccauccccaccaacuucacaaucagcgugaccacagagauccugcccgugagcaugaccaagacaagcguggacugcacaauguauaucuguggcgauagcaccgagugcuccaaccugcugcugcaguacggcuccuuuuguacccagcugaaucgcgcccugacaggcaucgcuguggagcaggauaagaacacacaggagguguucgcccaggugaagcagaucuacaagaccccacccaucaaggacuuuggcggcuucaauuuuucccagauccugcccgauccuagcaagccuuccaagagaucuuuuaucgaggaccugcuguucaacaaggugacccuggcugaugccggcuucaucaagcaguauggcgauugccugggcgacaucgcugcuagggaccugaucugugcucagaaguuuaauggccugaccgugcugccuccacugcugacagaugagaugaucgcucaguacacaagcgcccugcuggcuggaaccaucacauccggauggaccuucggcgcuggagcugcccugcagaucccauuugccaugcagauggcuuauagauucaacggcaucggcgugacccagaaugugcuguacgagaaccagaagcugaucgccaaucaguuuaacuccgcuaucggcaagauccaggacagccugagcagcacagcuuccgcccugggcaagcugcaggauguggugaaucagaacgcucaggcccugaauacccuggugaagcagcugucuagcaacuucggcgcuaucuccucugugcugaaugauauccugagccggcuggacccuccagaggcugaggugcagaucgaccggcugaucacaggcaggcugcagucccugcagaccuaugugacacagcagcugaucagagcugccgagauccgcgcuucugccaaucuggcugccaccaagauguccgagugcgugcugggccagucuaagcgcguggacuuuuguggcaagggcuaucaccugaugucuuucccacagagcgccccacacggagugguguuucugcacgugaccuacgugccugcccaggagaagaacuucaccacagcuccagccaucugccacgauggcaaggcccacuuuccacgggagggcguguucgugagcaacggcacccacugguuugugacacagaggaauuucuacgagccccagaucaucaccacagacaauaccuucgugagcggcaacugugacguggucaucggcaucgugaacaauaccguguaugauccucugcagccagagcuggacucuuuuaaggaggagcuggauaaguacuucaagaaucacaccagccccgacguggaucugggcgacaucuccggcaucaaugcuucuguggugaacauccagaaggagaucgaccgccugaacgagguggccaagaaucugaacgagagccugaucgaucugcaggagcugggcaaguaugagcaguacaucaaguggcccugguauaucuggcugggcuucaucgccggccugaucgccaucgugauggugaccaucaugcugugcuguaugacaagcugcuguuccugccugaagggcugcuguucuuguggcagcugcuguaaguuugaugaggacgauagcgagccugugcugaagggcgugaagcugcacuacaccugauaauaggcuggagccucgguggccaugcuucuugccccuugggccuccccccagccccuccuccccuuccugcacccguacccccguggucuuugaauaaagucugagugggcggcaaaaaaaaaaaaaaaaaaaaaaaaaaaaaaaaaaaaaaaaaaaaaaaaaaaaaaaaaaaaaaaaaaaaaaaaaaaaaaaaaaaaaaaaaaaaaaaaaaaa

SEQ ID NO: 18 - RNA, 990 nt, Artificial Sequence
  mRNA
ggggaaauaagagagaaaagaagaguaagaagaaauauaagagccaccauggacuggaccuggauccuguuccuggucgccgcugccacccgggugcacagcagagugcagcccaccgagucuaucgugcgguuucccaacaucaccaaccucuguccuuucggcgaagucuuuaacgccacaagauucgccagcguuuacgccuggaauaggaaaagaaucagcaauugcguggccgacuacagcgugcuguacaacagcgccucuuucagcaccuucaaguguuacggaguguccccuacaaagcugaacgaccugugcuucacaaacguguacgcugauucuuuugugauuagaggcgacgaggugcggcagaucgccccuggccagaccggcaacaucgcugauuacaacuauaagcugccugacgacuucaccggaugugugaucgccuggaacagcaauaaccuggacuccaaggugggaggcaauuacaacuaccuguaccggcuguucagaaaguccaaccugaagcccuucgaaagagauaucagcacagagaucuaccaggccggcagcaccccaugcaacggcgugaagggcuucaacugcuacuucccccugcagagcuacggcuuucagccuaccuacggcguggguuaucaaccauacagaguggugguccugagcuucgagcugcugcacgccccugccaccgugugcggcccuaagaaaucuacaaaucuggugaaaaacaagugcgugaacuucugauaauaggcuggagccucgguggccaugcuucuugccccuugggccuccccccagccccuccuccccuuccugcacccguacccccguggucuuugaauaaagucugagugggcggcaaaaaaaaaaaaaaaaaaaaaaaaaaaaaaaaaaaaaaaaaaaaaaaaaaaaaaaaaaaaaaaaaaaaaaaaaaaaaaaaaaaaaaaaaaaaaaaaaaaa

SEQ ID NO: 19 - RNA, 4077 nt, Artificial Sequence
  mRNA
ggggaaauaagagagaaaagaagaguaagaagaaauauaagagccaccauguucguguuucuggugcugcugccccuggugagcucccagugcgugaauuucaccaccagaacccagcugccaccugccuauaccaacaguuucaccagaggcguguacuaccccgauaagguguuuagauccagcgugcugcacagcacccaagaccuguuucugcccuucuucagcaacgugaccugguuccacgcuauccacgugagcggcaccaacggcacuaagagguucgccaauccugugcugccuuucaacgacggcguauauuuugccagcaccgaaaagagcaacaucaucagaggauggaucuucggaaccacccuggacagcaagacccagagccugcugaucgugaacaacgccaccaacguggugaucaaggugugugaauuccaauucugcaacgacccuuuccugggagucuacuaccacaagaacaacaagagcuggauggaauccgaguucagaguguacucuagcgcuaauaacugcaccuuugaguacgugagccagccauuccugauggaccuggaaggcaagcaaggcaacuucaagaauuugcgggaauucgucuucaaaaacaucgacggcuacuucaagaucuacagcaagcacacccccaucaaccuggucagaggacugccucaaggcuuuucugcucuggaaccucuaguugaccugccuaucggcauuaacaucacaagauuccagacacugcacaucagcuaccugaccccuggagauagcucuagcggauggacagccggcgcugccgccuacuacgugggauaucugcagcccagaacauuccugcugaaauacaacgagaacgguacaaucaccgacgccguggacugcgcccuggacccucugucugagacaaagugcacgcugaaguccuucacaguggaaaagggcaucuaucagaccagcaauuuccgcgugcagccuaccgagagcauagugcgguuccccaacaucaccaaccuguguccuuuuggcgagguguucaaugccacacgguucgccuccguguacgccuggaacagaaagcggaucagcaauugcguggccgacuacuccgugcuguacaacagcgccagcuucagcaccuucaagugcuacggcguguccccuacgaaacugaacgaucugugcuucaccaacguguacgccgacagcuucgugauccgaggcgacgaggugagacagaucgccccuggccagaccggcaacaucgccgauuacaacuacaagcugccugacgacuucaccggcugcgugaucgccuggaauagcaacaaccuggauucuaaagugggcggcaauuacaacuaccuguacagacuguucagaaagucgaaccugaaaccuuucgagagagauaucucuaccgagaucuaccaggccggcagcacccccugcaauggcgucaaaggcuucaacuguuacuucccucugcagagcuacggcuuucagccaaccuacggcgucggcuaccagccauacagagugguagugcucagcuucgagcugcugcaugcccccgccacaguuuguggcccuaagaaaagcacaaaucuggugaagaacaagugcgugaacuucaacuucaacggccugacaggcaccggagugcucaccgagagcaacaaaaaguuccugccuuuccagcaguuugggagagauaucgcagacaccacagaugccgugcgggacccccagacccucgaaauccuggacaucacaccuuguagcuuuggaggcgugucugugauuacaccuggcacaaacacaagcaaccagguggcugugcuguaccaaggcgucaacugcaccgaagugcccguggcuauccacgccgaccagcugaccccgaccuggcggguguacagcacaggcaguaauguguuucagacccgggccggcugucugaucggagccgagcacgugaacaacagcuacgagugcgacauccccaucggcgccggcaucugcgccucuuaucagacacagacaaacagccccggaucugcuggcagcguugcuagccagucuaucauugccuacaccaugucccugggcguggagaauucuguggcuuacuccaacaauucuaucgccauccccaccaacuucacaaucagcgugaccacagagauccugcccgugagcaugaccaagacaagcguggacugcacaauguauaucuguggcgacagcaccgagugcuccaaccugcugcugcaguacggcuccuuuuguacccagcugaaucgcgcccugacaggcaucgcuguggagcaggacaagaacacacaggagguguucgcccaggugaagcagaucuacaagaccccacccaucaaggacuuuggcggcuucaauuuuucccagauccugcccgaucccagcaagccuuccaagagaucuuuuaucgaggaccugcuguucaacaaggugacccuggccgaugccggcuucaucaagcaguauggcgauugccugggcgacaucgcugccagggaccugaucugugcucagaaguucaauggccugaccgugcugccuccacugcugacagacgagaugaucgcucaguacacaagcgcccugcuggcuggaaccaucacauccggcuggaccuucggcgcuggagcugcccugcagaucccauuugccaugcagauggcuuacagauucaacggcaucggcgugacccagaaugugcuguacgagaaccagaagcugaucgccaaucaguucaacuccgcuaucggcaagauccaggacagccugagcagcacagcuuccgcccugggcaagcugcaggauguggugaaucagaacgcucaggcccugaauacccuggugaagcagcugucgagcaacuucggcgcuaucuccucugugcugaacgauauccugagccggcuggacccuccagaggcggaggugcagaucgaccggcugaucacaggcaggcugcagucccugcagaccuaugugacacagcagcugaucagagcugccgagauccgcgcuucugccaaucuggcugccaccaagauguccgagugcgugcugggccagucgaagcgcguggacuuuuguggcaagggcuaucaccugaugucuuucccacagagcgccccacacggagugguguuucugcacgugaccuacgugccugcccaggagaagaacuucaccacagcuccagccaucugccacgauggcaaggcccacuuuccacgggagggcguguucgugagcaacggcacccacugguuugugacacagaggaauuucuacgagccccagaucaucaccacagacaauaccuucgugagcggcaacugcgacguggucaucggcaucgugaacaauaccguguacgauccucugcagccagagcuggacucuuucaaggaggagcuggacaaguacuucaagaaucacaccagccccgacguggaucugggcgacaucuccggcaucaaugcuucuguggugaacauccagaaggagaucgaccgccugaacgagguggccaagaaucugaacgagagccugaucgaucugcaggagcugggcaaguacgagcaguacaucaaguggcccugguauaucuggcugggcuucaucgccggccugaucgccaucgugauggugaccaucaugcugugcuguaugacaagcugcuguuccugccugaagggcugcuguucuuguggcagcugcugcaaguucgacgaggacgacagcgagccugugcugaagggcgugaagcugcacuacaccugauaauaggcuggagccucgguggccaugcuucuugccccuugggccuccccccagccccuccuccccuuccugcacccguacccccguggucuuugaauaaagucugagugggcggcaaaaaaaaaaaaaaaaaaaaaaaaaaaaaaaaaaaaaaaaaaaaaaaaaaaaaaaaaaaaaaaaaaaaaaaaaaaaaaaaaaaaaaaaaaaaaaaaaaaa